European Patent Specification EP 3 764 773 B1, published July 15, 2026. Title: Brassica plant resistant to Plasmodiophora brassicae (clubroot). Applicant: BASF Agricultural Solutions Seed US LLC. The sequence listing filed with the application follows.

SEQUENCE LISTING (12 sequences)

SEQ ID NO: 1 - DNA, 3623 bp, Brassica napus
atggctctctcattagcttcttctccttcctcttgtcgcacttggttgtacgatgttttccctagcttcagtggggtagacgttcgtgttactttcctcagccacttgttgaaggagtttgacaaaaagttgatcactgctttcaaagacaacgagatcgagagaagtcgatcactggatcccgagcttaaacaagccattaaagattcgaggatcgcagtggttatcttctcccaaaactatgcctcttcaagctggtgtcttaatgagttgttagagatagtcaagtgtggtcaaatggtgatacctgttttctaccggttggatccttcccatgtgaggaaacaaaccggtgactttggtaagttctttgaagaaacatgcaacaacaaaacagaggaagagaaaatacagtggaggagagctttgaccgatgtagccaatactctcgggtatcattcagtaaactggggtaacgaagctgcaatgattgaagaaatcgccaatgatgttttggataaactacttttaacttcatcgaaggattcagagaactttgtgggcatcgaagatcatgttgcaaaactgagtgtattgctgcagttggacgcggaggaagtgaggatggttggtttatggggttcctcagggatcggcaagactacaattgcaagagttctgtttcaacgactttctcgacacttccgaggtagcattttcatagacagggctttcgtatctaagactatggaaattttcaaggcagctaatccggacgactataacatgaagctgcatttgcaaagaaatttcctatctgaaatcttaggtaaaggagacataaagataaatcatttgagtgcagttggggagaggctgaagaatcagaaagttcttattttcattgatgattttgatgatcaagttgtgctagaagccttggttggtcaaactcaatggtttggaagtgggagcagaatcgttgtggttacaaatgataagcagtatctaagggcccatgggattaatcacatttacaaggtctgtctcccaactaaaaagctagctgttgagatgttatgtcgatctgctttcaggaaaaaggctgcacctgaaggttttgaggagcttgtagctaaagttacaggacttgctggtagtcttcctttaggtcttaatgttttgggttcatatctacggggaagggacaaggagtactggatggatttgttgccaaggcttcagaatggtttagatgggaaaattgagaagacattgagagtcagctacgatggattaacaagcgaagaagataaagcgttatttcgccatattgcatgccttttccagtgggaaaaagtcacatacctgaagttgctgctcgctgatagtgggttgagtgttacggttgggctggaaaacctagctgataagtccctcattcatgtaagagaggattatgtgaagatgcaccgtttgttagaagagatgggtagacgtattgttaggcttgacgagcctgaaaaacgagaatttctggtggacgcacaagatatctgtgatgtactcagtcaagacactggtactcataagatattgggtataaaattgaatattgatgagattgatgaactgaatgtgcatgagaatgccttcaaagggatgcgcaatctgcgtttcctggaaattcactcacaaaaccgtcatgagtttggaaacgaagaagttagaattcacttacctgaaaacttcgactatttgcctcctaaacttaaaatattggattggtatgaatatccaatgagatgtctgccttctaagtttcgtcctgaaaaactcgtcaagctcaaaatggtgaatagcaagctcgagaagctgtgggaagggattgtgtcgcttacatgtcttaaaaagatgaatatgtcgggatctcaaaacttgatagaaatgccagatctttcaaaggccaccaatctggagacactatatcttgaggattgctttagtttggtcaagcttccttcctctattccacaccccaacaaactgacgacattaatcttgaagaactgtcgaaatgtggagactattccaattggcattagcctcaaatctcttaaaaacctacgtactgatggttgctcacggatgaggacttttccccaaatctcaagcaccatcgaagatgtctacataggcgcaacatccattgaagaaataccttcaaatttgagtttgtgtttcgagaatctccatacctttacgatgcacagcccaaagaaactatgggaaagagtgcagcttcttactctcctcacgacgatcatgtctccctctttgtggtatctggatctctcggataaccctggcttggtggagcttccttcttcatttaagaatctccataacctgaggagattggaaattagaaactgcgtaaatctggaaactcttcccaccggaatcaacctcggatctctcaaaatcctagatctcaggggatgctcacggttgaggacttttcctgatatctcaacccacatcacacatctttatctaagcggaacagggattgaagagattccttgttcgattgagaaattctccaggcttggctccctacatatgaacggatgcaacaatttggaatatgtaaacctaaacctttttaaactcaaacatcttcacgaagtcgacttttcagactgcaagtgcttaaacttggatcaagaagctctgtttcaaaagaaaacatattcagtttgtcaactgaagttgtcaggtgaagaagtgccttcatatttcacgcaccgtactactggaacctcctcctctctcaccattcctctacttcacagctgtatctcacaatcattcctccgattcagggcttgtattgtgtttgattcggacaaggacaatgagtcatatagcagatgtgcctttagattcaaaggcagttttcggaactgctctgattcctataatcaggcacaagacttctgcgcagtcacggatgattataagatccgttcatataagaaggatggttgtctgcttgtattagactaccagatgtctcaaatccctttagaaatgaacttcgatggcctggatctgaagattcatattgattattgtcgttctgctaaaataaaaggatggggtatacgaatcttagaggaggactgttcatcggcagacaaccgacttggttatccaaacattctaccacatgtttttgaagccgatgaatgcaatgaggctgatttcgtgaataaacttttgattgtgttaggttgtaacgcagagcatctaaaattaggaattaagagagattcccatccaacttgcttgtggatcttagtatgcggagaagcagtgcctctttttctatcagagattgctcctgcacagctcaggggaggtctcaacattgtattccaactcatggtcacaattggaatcctaatagccaaccttgtcaactacttcactgccaccgttcaccctaacggatggcgaatcgccctcggtggagccgcaatccccaccgttatcctagtcttcggttcactgatcatctgcgagactcccacgagcttcatagagcgcaagtgttg

SEQ ID NO: 2 - DNA, 4749 bp, Brassica napus
gccagctatttaggtgacactatagaatactcaagctatgcatcaagcttggtaccgagctcggatccactagtaacggccgccagtgtgctggaattcgcccttttgcgctacactccaatctgacaatttatatggactaacattcttcagaagatcaatcaccaagtccttcttttccttcatattatttttgctcctatctctatggctctctcattagcttcttctccttcctcttgtcgcacttggttgtacgatgttttccctagcttcagtggggtagacgttcgtgttactttcctcagccacttgttgaaggagtttgacaaaaagttgatcactgctttcaaagacaacgagatcgagagaagtcgatcactggatcccgagcttaaacaagccattaaagattcgaggatcgcagtggttatcttctcccaaaactatgcctcttcaagctggtgtcttaatgagttgttagagatagtcaagtgtggtcaaatggtgatacctgttttctaccggttggatccttcccatgtgaggaaacaaaccggtgactttggtaagttctttgaagaaacatgcaacaacaaaacagaggaagagaaaatacagtggaggagagctttgaccgatgtagccaatactctcgggtatcattcagtaaactggtacggttttatgcttcttttgaataaaggttagacttctggttgctagggggtgatattatctttcttattgttaggggtaacgaagctgcaatgattgaagaaatcgccaatgatgttttggataaactacttttaacttcatcgaaggattcagagaactttgtgggcatcgaagatcatgttgcaaaactgagtgtattgctgcagttggacgcggaggaagtgaggatggttggtttatggggttcctcagggatcggcaagactacaattgcaagagttctgtttcaacgactttctcgacacttccgaggtagcattttcatagacagggctttcgtatctaagactatggaaattttcaaggcagctaatccggacgactataacatgaagctgcatttgcaaagaaatttcctatctgaaatcttaggtaaaggagacataaagataaatcatttgagtgcagttggggagaggctgaagaatcagaaagttcttattttcattgatgattttgatgatcaagttgtgctagaagccttggttggtcaaactcaatggtttggaagtgggagcagaatcgttgtggttacaaatgataagcagtatctaagggcccatgggattaatcacatttacaaggtctgtctcccaactaaaaagctagctgttgagatgttatgtcgatctgctttcaggaaaaaggctgcacctgaaggttttgaggagcttgtagctaaagttacaggacttgctggtagtcttcctttaggtcttaatgttttgggttcatatctacggggaagggacaaggagtactggatggatttgttgccaaggcttcagaatggtttagatgggaaaattgagaagacattgagagtcagctacgatggattaacaagcgaagaagataaagcgttatttcgccatattgcatgccttttccagtgggaaaaagtcacatacctgaagttgctgctcgctgatagtgggttgagtgttacggttgggctggaaaacctagctgataagtccctcattcatgtaagagaggattatgtgaagatgcaccgtttgttagaagagatgggtagacgtattgttaggcttgacgagcctgaaaaacgagaatttctggtggacgcacaagatatctgtgatgtactcagtcaagacactgtaagttatctcttatgttcgtgctcctttcagtcaataaataagatttagagcatgccattttataagcaaaactaatacttgatattatataattttcagggtactcataagatattgggtataaaattgaatattgatgagattgatgaactgaatgtgcatgagaatgccttcaaagggatgcgcaatctgcgtttcctggaaattcactcacaaaaccgtcatgagtttggaaacgaagaagttagaattcacttacctgaaaacttcgactatttgcctcctaaacttaaaatattggattggtatgaatatccaatgagatgtctgccttctaagtttcgtcctgaaaaactcgtcaagctcaaaatggtgaatagcaagctcgagaagctgtgggaagggattgtggtaagttttgagaatagtttgtgatgttatttgtagtaagactaatctttattttattttttggatgacaatcttgttctactgagctcatgtgttctgttcctttttttttttgttgagtacagtcgcttacatgtcttaaaaagatgaatatgtcgggatctcaaaacttgatagaaatgccagatctttcaaaggccaccaatctggagacactatatcttgaggattgctttagtttggtcaagcttccttcctctattccacaccccaacaaactgacgacattaatcttgaagaactgtcgaaatgtggagactattccaattggcattagcctcaaatctcttaaaaacctacgtactgatggttgctcacggatgaggacttttccccaaatctcaagcaccatcgaagatgtctacataggcgcaacatccattgaagaaataccttcaaatttgagtttgtgtttcgagaatctccatacctttacgatgcacagcccaaagaaactatgggaaagagtgcaggtatgtatgtagttccaaactttgtgtgtttctccaatctgttttacgttatagatattagataatggtgcaaatgaaactaaggttatattgtatttatcggagggaagaagagtagcgctgaatatgattttgtgtatttggttcagcttcttactctcctcacgacgatcatgtctccctctttgtggtatctggatctctcggataaccctggcttggtggagcttccttcttcatttaagaatctccataacctgaggagattggaaattagaaactgcgtaaatctggaaactcttcccaccggaatcaacctcggatctctcaaaatcctagatctcaggggatgctcacggttgaggacttttcctgatatctcaacccacatcacacatctttatctaagcggaacagggattgaagagattccttgttcgattgagaaattctccaggcttggctccctacatatgaacggatgcaacaatttggaatatgtaaacctaaacctttttaaactcaaacatcttcacgaagtcgacttttcagactgcaagtgcttaaacttggatcaagaagctctgtttcaaaagaaaacatattcagtttgtcaactgaagttgtcaggtgaagaagtgccttcatatttcacgcaccgtactactggaacctcctcctctctcaccattcctctacttcacagctgtatctcacaatcattcctccgattcagggcttgtattgtgtttgattcggacaaggacaatgagtcatatagcagatgtgcctttagattcaaaggcagttttcggaactgctctgattcctataatcaggcacaagacttctgcgcagtcacggatgattataagatccgttcatataagaaggatggttgtctgcttgtattagactaccagatgtctcaaatccctttagaaatgaacttcgatggcctggatctgaagattcatattgattattgtcgttctgctaaaataaaaggatggggtatacgaatcttagaggaggactgttcatcggcagacaaccgacttggttatccaaacattctaccacatgtttttgaagccgatgaatgcaatgaggctggtgaatgtgggaggcaaatgatgtagtgacggaaagaagcgggtaaaggcattaatcatgaacttatcacagtattttctatatcataatttcttgtactgagacttttttttctttttctgcagatttcgtgaataaacttttgattgtgttaggttgtaacgcagagcatctaaaattaggaattaagagagattcccatccaacttgcttgtggatcttagtatgcggagaagtaagagcacaaaattgtgggaaggagtagtgcatgtatgttttcttcaaccttccttcctttatactagttcttacaaaaatggttatgcctggcagatctctagaaatgacctaacattattgtgtgtaccttaaattctcaggcagtgcctctttttctatcagagattgctcctgcacagctcaggggaggtctcaacattgtattccaactcatggtcacaattggaatcctaatagccaaccttgtcaactacttcactgccaccgttcaccctaacggatggcgaatcgccctcggtggagccgcaatccccaccgttatcctagtcttcggttcactgatcatctgcgagactcccacgagcttcatagagcgcaagtgttgaaaccagcgagtcgtccacctttaatcattggaatgcttctacagcttttccagcagtttagtggaatcaatgctattatgttctacgcaccggttttaagggcgaattctgcagatatccatcacactggcggccgctcgagcatgcatctagagggcccaattcgccctatagtgagtcgtatacaatcactgc

SEQ ID NO: 3 - protein, 1207 aa, Brassica napus
MALSLASSPSSCRTWLYDVFPSFSGVDVRVTFLSHLLKEFDKKLITAFKDNEIERSRSLDPELKQAIKDSRIAVVIFSQNYASSSWCLNELLEIVKCGQMVIPVFYRLDPSHVRKQTGDFGKFFEETCNNKTEEEKIQWRRALTDVANTLGYHSVNWGNEAAMIEEIANDVLDKLLLTSSKDSENFVGIEDHVAKLSVLLQLDAEEVRMVGLWGSSGIGKTTIARVLFQRLSRHFRGSIFIDRAFVSKTMEIFKAANPDDYNMKLHLQRNFLSEILGKGDIKINHLSAVGERLKNQKVLIFIDDFDDQVVLEALVGQTQWFGSGSRIVVVTNDKQYLRAHGINHIYKVCLPTKKLAVEMLCRSAFRKKAAPEGFEELVAKVTGLAGSLPLGLNVLGSYLRGRDKEYWMDLLPRLQNGLDGKIEKTLRVSYDGLTSEEDKALFRHIACLFQWEKVTYLKLLLADSGLSVTVGLENLADKSLIHVREDYVKMHRLLEEMGRRIVRLDEPEKREFLVDAQDICDVLSQDTGTHKILGIKLNIDEIDELNVHENAFKGMRNLRFLEIHSQNRHEFGNEEVRIHLPENFDYLPPKLKILDWYEYPMRCLPSKFRPEKLVKLKMVNSKLEKLWEGIVSLTCLKKMNMSGSQNLIEMPDLSKATNLETLYLEDCFSLVKLPSSIPHPNKLTTLILKNCRNVETIPIGISLKSLKNLRTDGCSRMRTFPQISSTIEDVYIGATSIEEIPSNLSLCFENLHTFTMHSPKKLWERVQLLTLLTTIMSPSLWYLDLSDNPGLVELPSSFKNLHNLRRLEIRNCVNLETLPTGINLGSLKILDLRGCSRLRTFPDISTHITHLYLSGTGIEEIPCSIEKFSRLGSLHMNGCNNLEYVNLNLFKLKHLHEVDFSDCKCLNLDQEALFQKKTYSVCQLKLSGEEVPSYFTHRTTGTSSSLTIPLLHSCISQSFLRFRACIVFDSDKDNESYSRCAFRFKGSFRNCSDSYNQAQDFCAVTDDYKIRSYKKDGCLLVLDYQMSQIPLEMNFDGLDLKIHIDYCRSAKIKGWGIRILEEDCSSADNRLGYPNILPHVFEADECNEADFVNKLLIVLGCNAEHLKLGIKRDSHPTCLWILVCGEAVPLFLSEIAPAQLRGGLNIVFQLMVTIGILIANLVNYFTATVHPNGWRIALGGAAIPTVILVFGSLIICETPTSFIERKC

SEQ ID NO: 4 - DNA, 3729 bp, Brassica napus
atggctctctcattagcttcttctccttcctcttctcgcacttggttgtacgatgttttccctagcttcagtggggtagacgtccgtgttactttcctcagccacttgttgaaggagtttgacaaaaagttgatcactgctttcaaagacaacgagatcgagagaagtcgatcactggatcccgagcttaaacaagccattaaagattcgaggatcgcggtggttatcttctcccaaaactatgcctcttcaagctggtgtcttaatgagttgttagagatagtcaagcgtggtcaaatggtgatacctgttttctaccggttggatccttcccacgtgaggaaacaaaccggtgacttcgggaaaatatttgaagaaacatgcaagaatcaaaaagaggaagtgataataattcaatggaggagagctttgaccgatgtagccaatacactcgggtatcattcagtaaactggggtaacgaagctgcaatgattgaagaaatcgccaatgatgttttggataaactacttttaacttcatcgaaggattcagagaactttgtgggcatcgaagatcatatcgcagaactgagtgtactgttgcagttggacgcggaggaagtgaggatggttggtttatggggttcctcagggatcggcaagactacaattgcaagagttctgtttcaacgactttctcgacacttccgaggtagcattttcatagacagggctttcgtatctaagactatggaaattttcaaggcagctaatccggacgactataacatgaagctgcatttgcaaagaaatttcctatctgaaatcttaggtaaaggagacataaagataaatcatttgagtgcagttggggagaggctgaagaatcagaaagttcttattttcattgatgattttgatgatcaagttgtgctagaagccttggttggtcaaactcaatggtttggaagtgggagcagaatcgttgtggttacaaatgataagcagtatctaagggcccatgggattaatcacatttacgaggtctgtctcccaactggaaacctagctgttgagatgttatgtcgatatgctttcaggaaaaaggctgcacctgaaggttttgaggagcttgtagctaaagttacaggacttgctggtagtcttcctttaggtcttaatgttttgggttcatctctacggggaagggacaaggagtactggatggatttgttgccaaggcttcggaattgtttagatgggaaaattgagaagacattgagagtcagctacgatggattaacaagcgaagaagataaagccttatttcgccatatcgcatgccttttcaatggtgcaacagtcacatacctgaagttggtgctcactgatagtgggttgagtgttaatgtggggctggaaaacctagctgataagtccctcattcatgaaagagaggattatgtggagatgcaccgtttgttagaagagatgggtagacgtattgttaggcttgaggagcctgaaaaacgagaatttctggtggacgcacaagatatctgtgatgtactcagtcaagacactggtactcataagatattgggtataaaattgaatattgatgagattgatgaactgaatgtgcatgagaatgccttcaaagggatgcgcaatctgcgtttcctggaaattcactcaaaaaagcgttatgtgtttggaaaggaagaagtaccaattcacttacctgaaaacttcgactatttgcctccaaaacttaaaatattggattggtatgaatatccaatgagatgtctgccttctaagtttcgtcctgaaaaactcgtcaagctcaaaatggtgaatagcaagctcgagaagctgtggaaagggattgtgtcgcttacatgtcttaataagatggatatgtcggcatctcaaaacttgatagaaatgccagatctttcaaaggccaccaatctggagacacttaaacttcggaattgctatagtttggtcaagcttccttcctctattccacatcccaacaaactgacgacattaaacttgaagaactgtcgaaatctggagactattccaattggcattagcctcaaatctctcaaaaacctaaatactaaaggatgctcacggatgaggatttttccccaaatctcaaccagcatcgtagatgtcgacatagccgcaacatccattgaagaaataccttcaaatttgagtttgtgtttcgagagtctccatacctttacgatgcacagcccaaagaaactatgggaaagagtgcagcttcttactctcctcacgacgatcatgtctccctctttgtggtatctggatctctcggataacccaggcttggtggagcttccttcttcatttaagaatctccataacttgcagatattgaaaattagtaactgcgtaaatctggaaactcttcccaccggaatcaacctcggatctctctggcaactagatctcagtggatgctcaaggttgaggacttttcctgatatctcaaccaacatcatagttctcgatctcagcgaaacagccatcgaagagattccttgttggattgagaaattctctaaccttaactcccttaggatgaagggatgcaacaatttggaatatgtaaacctaaacatttctaaactcaaacatcttcagaaagtagacttttcagactgcaagtcattgactggagctagcttgaataatcgtccaagagaaagtgccttgagttattaccacatatgctacattggtatcgatttcaccaagtgcttaaacttggatcaagaagctctgtttcaaaagaaaacatattttggttgtcatctgaagttgtcaggtgaagaagtgccttcatatttcactcaccgtactactggaacctcctcctctctcaccattcctttacttcacagctgtctctcacaaccattcctcctattcagggcttgtattgtgtttgattcggacaaggagacatatagcgattgtgtctttagattcaaaggcagttttcggaactgctctgattcctataatcaggcacaagacttctgcgcagtcacggatgattatgagatcaattcatatgagaaggatggttgtctgtttgtattagactaccagatgtctcaaatccctttagaaatgaacttcgatcgcctggatctgaagattcatattgttgattgttttaatgatgctaaaataaaaggatggggtatacgaatcttagaggaggactgttcatcggcagacaaccgacttggttatccaaacattctaccacatgtttttgaagccgatgaatgcaatatgaggctggtgaatgtggaggcaaatgatgcagtgacggaaagaagcggtatgcggagaagtaagagcacaatattgtgggaaggagtagtgcatgcagtgcctctttttctatcagagattgctcctgcacagctcaggggaggtctcaacattgtattccaactcatggtaacaattggaatcctaatagccaaccttgtcaactacttcactgccaccgttcaccctaacggatggcgaatcgccctcggtggagctgcaatccccgcggttatcctcctcttgggttcactgatcatctgtgagacccccacgagcctcatagagcgcaacaaaaacgaagaaggcagagaaactctaaggaaaatcagagga

SEQ ID NO: 5 - DNA, 4492 bp, Brassica napus
atggctctctcattagcttcttctccttcctcttctcgcacttggttgtacgatgttttccctagcttcagtggggtagacgtccgtgttactttcctcagccacttgttgaaggagtttgacaaaaagttgatcactgctttcaaagacaacgagatcgagagaagtcgatcactggatcccgagcttaaacaagccattaaagattcgaggatcgcggtggttatcttctcccaaaactatgcctcttcaagctggtgtcttaatgagttgttagagatagtcaagcgtggtcaaatggtgatacctgttttctaccggttggatccttcccacgtgaggaaacaaaccggtgacttcgggaaaatatttgaagaaacatgcaagaatcaaaaagaggaagtgataataattcaatggaggagagctttgaccgatgtagccaatacactcgggtatcattcagtaaactggtacggttttatgcatcattcattcttttgagtaaaggttagacttctggttgctagggggtgatattatatttcttaatgttaggggtaacgaagctgcaatgattgaagaaatcgccaatgatgttttggataaactacttttaacttcatcgaaggattcagagaactttgtgggcatcgaagatcatatcgcagaactgagtgtactgttgcagttggacgcggaggaagtgaggatggttggtttatggggttcctcagggatcggcaagactacaattgcaagagttctgtttcaacgactttctcgacacttccgaggtagcattttcatagacagggctttcgtatctaagactatggaaattttcaaggcagctaatccggacgactataacatgaagctgcatttgcaaagaaatttcctatctgaaatcttaggtaaaggagacataaagataaatcatttgagtgcagttggggagaggctgaagaatcagaaagttcttattttcattgatgattttgatgatcaagttgtgctagaagccttggttggtcaaactcaatggtttggaagtgggagcagaatcgttgtggttacaaatgataagcagtatctaagggcccatgggattaatcacatttacgaggtctgtctcccaactggaaacctagctgttgagatgttatgtcgatatgctttcaggaaaaaggctgcacctgaaggttttgaggagcttgtagctaaagttacaggacttgctggtagtcttcctttaggtcttaatgttttgggttcatctctacggggaagggacaaggagtactggatggatttgttgccaaggcttcggaattgtttagatgggaaaattgagaagacattgagagtcagctacgatggattaacaagcgaagaagataaagccttatttcgccatatcgcatgccttttcaatggtgcaacagtcacatacctgaagttggtgctcactgatagtgggttgagtgttaatgtggggctggaaaacctagctgataagtccctcattcatgaaagagaggattatgtggagatgcaccgtttgttagaagagatgggtagacgtattgttaggcttgaggagcctgaaaaacgagaatttctggtggacgcacaagatatctgtgatgtactcagtcaagacactgtaagttatctcttatgttcgtgctcctttcagtcaataaataagatttagagcatgccattttataagcaaaactaatacttgatattatataattttcagggtactcataagatattgggtataaaattgaatattgatgagattgatgaactgaatgtgcatgagaatgccttcaaagggatgcgcaatctgcgtttcctggaaattcactcaaaaaagcgttatgtgtttggaaaggaagaagtaccaattcacttacctgaaaacttcgactatttgcctccaaaacttaaaatattggattggtatgaatatccaatgagatgtctgccttctaagtttcgtcctgaaaaactcgtcaagctcaaaatggtgaatagcaagctcgagaagctgtggaaagggattgtggtaagttttgagaatagtttgtgatgttattagtagtaagactaatcttgattttattttttggatgacaatcttgttctactgagctcatgtgttttgttcctttttatttgttttgttgagtacagtcgcttacatgtcttaataagatggatatgtcggcatctcaaaacttgatagaaatgccagatctttcaaaggccaccaatctggagacacttaaacttcggaattgctatagtttggtcaagcttccttcctctattccacatcccaacaaactgacgacattaaacttgaagaactgtcgaaatctggagactattccaattggcattagcctcaaatctctcaaaaacctaaatactaaaggatgctcacggatgaggatttttccccaaatctcaaccagcatcgtagatgtcgacatagccgcaacatccattgaagaaataccttcaaatttgagtttgtgtttcgagagtctccatacctttacgatgcacagcccaaagaaactatgggaaagagtgcaggtatgtatgtagttccaaactttgtgtgtttctccaatctgttttacgttatagatattagataatggtgcaaatgaaactaaggttatattgtatttatcggagggaagaagagtagcgctgaatatgattttgtgtatttggttcagcttcttactctcctcacgacgatcatgtctccctctttgtggtatctggatctctcggataacccaggcttggtggagcttccttcttcatttaagaatctccataacttgcagatattgaaaattagtaactgcgtaaatctggaaactcttcccaccggaatcaacctcggatctctctggcaactagatctcagtggatgctcaaggttgaggacttttcctgatatctcaaccaacatcatagttctcgatctcagcgaaacagccatcgaagagattccttgttggattgagaaattctctaaccttaactcccttaggatgaagggatgcaacaatttggaatatgtaaacctaaacatttctaaactcaaacatcttcagaaagtagacttttcagactgcaagtcattgactggagctagcttgaataatcgtccaagagaaagtgccttgagttattaccacatatgctacattggtatcgatttcaccaagtgcttaaacttggatcaagaagctctgtttcaaaagaaaacatattttggttgtcatctgaagttgtcaggtgaagaagtgccttcatatttcactcaccgtactactggaacctcctcctctctcaccattcctttacttcacagctgtctctcacaaccattcctcctattcagggcttgtattgtgtttgattcggacaaggagacatatagcgattgtgtctttagattcaaaggcagttttcggaactgctctgattcctataatcaggcacaagacttctgcgcagtcacggatgattatgagatcaattcatatgagaaggatggttgtctgtttgtattagactaccagatgtctcaaatccctttagaaatgaacttcgatcgcctggatctgaagattcatattgttgattgttttaatgatgctaaaataaaaggatggggtatacgaatcttagaggaggactgttcatcggcagacaaccgacttggttatccaaacattctaccacatgtttttgaagccgatgaatgcaatatgaggctggtgaatgtggaggcaaatgatgcagtgacggaaagaagcgggtaaagggcattaatcatgaacttatcacagtattttctatatcataatttcttgtactgagactttttttttctttttctgcagatttcgtgaataaagttttgattgtgttaggttgtaacgcagagcatctaaaattaggaattaagagagtttcccatccaacttgcttgtggatcttagtatgcggagaagtaagagcacaatattgtgggaaggagtagtgcatgtatgttttcttcaaccttccttcctttatactagttcttacaaaaatggttatgcctggcagatctctagaaatgacctaactttattgtgtgtaccttaaattctcaggcagtgcctctttttctatcagagattgctcctgcacagctcaggggaggtctcaacattgtattccaactcatggtaacaattggaatcctaatagccaaccttgtcaactacttcactgccaccgttcaccctaacggatggcgaatcgccctcggtggagctgcaatccccgcggttatcctcctcttgggttcactgatcatctgtgagacccccacgagcctcatagagcgcaacaaaaacgaagaaggcagagaaactctaaggaaaatcagaggagttga

SEQ ID NO: 6 - protein, 1243 aa, Brassica napus
MALSLASSPSSSRTWLYDVFPSFSGVDVRVTFLSHLLKEFDKKLITAFKDNEIERSRSLDPELKQAIKDSRIAVVIFSQNYASSSWCLNELLEIVKRGQMVIPVFYRLDPSHVRKQTGDFGKIFEETCKNQKEEVIIIQWRRALTDVANTLGYHSVNWGNEAAMIEEIANDVLDKLLLTSSKDSENFVGIEDHIAELSVLLQLDAEEVRMVGLWGSSGIGKTTIARVLFQRLSRHFRGSIFIDRAFVSKTMEIFKAANPDDYNMKLHLQRNFLSEILGKGDIKINHLSAVGERLKNQKVLIFIDDFDDQVVLEALVGQTQWFGSGSRIVVVTNDKQYLRAHGINHIYEVCLPTGNLAVEMLCRYAFRKKAAPEGFEELVAKVTGLAGSLPLGLNVLGSSLRGRDKEYWMDLLPRLRNCLDGKIEKTLRVSYDGLTSEEDKALFRHIACLFNGATVTYLKLVLTDSGLSVNVGLENLADKSLIHEREDYVEMHRLLEEMGRRIVRLEEPEKREFLVDAQDICDVLSQDTGTHKILGIKLNIDEIDELNVHENAFKGMRNLRFLEIHSKKRYVFGKEEVPIHLPENFDYLPPKLKILDWYEYPMRCLPSKFRPEKLVKLKMVNSKLEKLWKGIVSLTCLNKMDMSASQNLIEMPDLSKATNLETLKLRNCYSLVKLPSSIPHPNKLTTLNLKNCRNLETIPIGISLKSLKNLNTKGCSRMRIFPQISTSIVDVDIAATSIEEIPSNLSLCFESLHTFTMHSPKKLWERVQLLTLLTTIMSPSLWYLDLSDNPGLVELPSSFKNLHNLQILKISNCVNLETLPTGINLGSLWQLDLSGCSRLRTFPDISTNIIVLDLSETAIEEIPCWIEKFSNLNSLRMKGCNNLEYVNLNISKLKHLQKVDFSDCKSLTGASLNNRPRESALSYYHICYIGIDFTKCLNLDQEALFQKKTYFGCHLKLSGEEVPSYFTHRTTGTSSSLTIPLLHSCLSQPFLLFRACIVFDSDKETYSDCVFRFKGSFRNCSDSYNQAQDFCAVTDDYEINSYEKDGCLFVLDYQMSQIPLEMNFDRLDLKIHIVDCFNDAKIKGWGIRILEEDCSSADNRLGYPNILPHVFEADECNMRLVNVEANDAVTERSGMRRSKSTILWEGVVHAVPLFLSEIAPAQLRGGLNIVFQLMVTIGILIANLVNYFTATVHPNGWRIALGGAAIPAVILLLGSLIICETPTSLIERNKNEEGRETLRKIRG

SEQ ID NO: 7 - DNA, 3585 bp, Brassica napus
atggctctctcattagcttcttctccttcctcttctcgcacttggttgtacgatgttttccctagcttcagtggggtagacgttcgtgttactttcctcagccacttgttgaaggagtttgacaaaaagttgatcactgctttcaaagacaacgagatcgagagaagtcgatcactggatcccgagctcaaacaagccattaaagattcgaggatcgcagtggttatcttctcccaaaactatgcctcttcaagctggtgtcttaatgagttgttagagatagtcaagcgtggtcaaatggtgatacctgttttctaccggttggatccttcccacgtgaggaaacaaaccggtgaatttgggaaaatatttgaagaaacatgcaagaatcaaaaagaggaagtgataataactcaatggaggagagctttgaccgatgtagccaatactctcgggtatcattcggtaaactggggtaacgaagctgcaatgattgaagaaatcgccaatgatgttttggataaactacttttaacttcatcgaaggattcagagaactttgtgggcatcgaagatcatcttgcagaactgagtgtattgctgcagttggacgcggaggaagtgaggatggttggtttatggggttcctcagggatcggcaagactacaattgcaagagttctgtttcaacgactttctcgacacttccgaggtagcattttcatagacagggctttcgtatctaagactatggaaattttcaaggaagctaatccggacgactataacatgaagctgcatttgcaaagaaatttcctatctgaaatcttaggtaaaggagacataaagataaatcatttgagtgcagttgaagagaggctgaagaatcagaaagttcttattttcattgatgattttgatgatcaagttgtgctagaagccttggttggtcaaactcaatggtttggaagtgggagcagaatcgttgtggttacaaatgataagcagtatctaagggcccatgggattaatcacatttacgaggtctgtctcccaactgaaaacctagctgttgagatgttatgtcgatctgctttcaggaaaaaggctgcacctgaaggttttgaggagcttgtagctaaagttacaggacttgctggtagtcttcctttaggtcttaatgttttgggttcatatctacggggaagggagaagaagtactggatggatttgttgccaaggcttcagaatggtttagatgggaaaattgagaagacattgagggtcagctacgatggattaacaagcgaagaagataaagcgttatttcgccatatcgcatgccttttccaatggaaaaaagtcacatacctgaagttgctgctcgctgatagtgggttgagtgttacggttgggctggaaaacctagctgataagtccatcattcatgtaagtacgaattatgtggtgatgcaccgtttgttagaagagatgggtagaggtattgttaggcttgacgagcctgaaaaacgagaatttctggtggacgcacaagatatctgtgatgtactcagtcaagacactggtactcataagatattgggtataaaattgaatattgatgagattgatgaactgaatgtgcatgagaatgccttcaaagggatgcgcaatctgcgtttcctggaaattcactcacaaaaccgtcatgagtttggaaacgaagaagttagaattcacttacctgaaaacttcgactatttgcctccaaaacttaaaatattggattggtttggatatccaatgagatgtctgccttctaagtttcgtcctgaaaaactcgtcaagctcaaaatggtgaatagcaagctcgagaagctgtgggaagggattgtgtcgcttacatgtcttaaagagatggatatgtcgggatctacaaacttgatagaaatgccagatctttcaaaggccaccaatctggagacacttaatgttggggcttgctatagtttggtgacttttccccaaatctcaagcaccatcgtagatgtcgacatagccggaacatccattgaagaaataccttcaaatttgagtttgtgtttcgagaatctccatacctttaagatgcacagcccaaagaaactatcggaaagagtgcagcttcttactctcctcacgccgatcatgtctccctctttgtggtatctgaatctctcggataaccctggcttggtggagcttccttcttcatttaagaatctccataaactggagagattgaaaattagaaactgcgtaaatctggaaactcttcccaccggaatcaacctcggatctctctcgagagtagatctaaggggatgctcacggttgagaacttttcctgatatctcaaccaacatcaaaaacctcgatctcagcgaaacagccattgaagagattccttgttggattgagaaattctccaggctttactccctacggatgaagggatgcaacaatttggaatatgtaaacctaaacatttctaaactcaaatatcttttcgaagtcgacttttcagactgcaagtcattgactggagctagctggaataatcgtccaagagaaagtgccttgagttattaccacagtttcgacattggtatcgatttcaccaagtgcttaaacttggatcaagaagctctgtttcaaaagaaaacatatttcggttgtcaactgaagttgtcaggtgaagaagtgccttcatatttcacgcaccgtactactggaacctcctcctctctcaccattcctttacttcacagctgtctctcacaaccattcctccgattcagggcttgcattgtgtttgattcgcacaatgagacatatagcaaatgtgtctttagattcaaaggcagttttcagaactgctctgattcctataatcaggcacaagacttctgcgcagtcacggaggattatttgatctattcatatgagaaggatggttgtctgtttgtattagactaccagatgtctcaaatccctttagaaatgaacttcgatggcctggatctgaagattcatattgttgattgttataatgctaaaataaaaggatggggtatacgaatcttagaggaggactgttcatcggcagacaaccgacttggttatccaaacattctaccacatgtttttgaagccgatgaatgcaatatgaggctggtgaatgtggaggcaaatgatgcagtgacggaaagaagcggtatgcggagaagtaagagcacaatattgtgggaaggagtagtgcatgcagtgcctctttttctatcagagattgttcctgcacagctcaagggaggtctcaacattgtattccaactcatggtcacaattggaatcctaatagccaacctggtcaactacttcactgccaccgttcaccctaacggatcgcgaatcgccctcggtggagctgcaatccccgcggttatcctcctcttgggttcactgatcatctgtgagacccccacgagcctcatagagcgcaacaaaaacgaagaaggcagagaaactctaaggaagatcagagga

SEQ ID NO: 8 - DNA, 4344 bp, Brassica napus
atggctctctcattagcttcttctccttcctcttctcgcacttggttgtacgatgttttccctagcttcagtggggtagacgttcgtgttactttcctcagccacttgttgaaggagtttgacaaaaagttgatcactgctttcaaagacaacgagatcgagagaagtcgatcactggatcccgagctcaaacaagccattaaagattcgaggatcgcagtggttatcttctcccaaaactatgcctcttcaagctggtgtcttaatgagttgttagagatagtcaagcgtggtcaaatggtgatacctgttttctaccggttggatccttcccacgtgaggaaacaaaccggtgaatttgggaaaatatttgaagaaacatgcaagaatcaaaaagaggaagtgataataactcaatggaggagagctttgaccgatgtagccaatactctcgggtatcattcggtaaactggtacggttttatgcatcattcattcttttgagtaaaggttagacttctggttgcttgggggtgatattatctttcttattgttaggggtaacgaagctgcaatgattgaagaaatcgccaatgatgttttggataaactacttttaacttcatcgaaggattcagagaactttgtgggcatcgaagatcatcttgcagaactgagtgtattgctgcagttggacgcggaggaagtgaggatggttggtttatggggttcctcagggatcggcaagactacaattgcaagagttctgtttcaacgactttctcgacacttccgaggtagcattttcatagacagggctttcgtatctaagactatggaaattttcaaggaagctaatccggacgactataacatgaagctgcatttgcaaagaaatttcctatctgaaatcttaggtaaaggagacataaagataaatcatttgagtgcagttgaagagaggctgaagaatcagaaagttcttattttcattgatgattttgatgatcaagttgtgctagaagccttggttggtcaaactcaatggtttggaagtgggagcagaatcgttgtggttacaaatgataagcagtatctaagggcccatgggattaatcacatttacgaggtctgtctcccaactgaaaacctagctgttgagatgttatgtcgatctgctttcaggaaaaaggctgcacctgaaggttttgaggagcttgtagctaaagttacaggacttgctggtagtcttcctttaggtcttaatgttttgggttcatatctacggggaagggagaagaagtactggatggatttgttgccaaggcttcagaatggtttagatgggaaaattgagaagacattgagggtcagctacgatggattaacaagcgaagaagataaagcgttatttcgccatatcgcatgccttttccaatggaaaaaagtcacatacctgaagttgctgctcgctgatagtgggttgagtgttacggttgggctggaaaacctagctgataagtccatcattcatgtaagtacgaattatgtggtgatgcaccgtttgttagaagagatgggtagaggtattgttaggcttgacgagcctgaaaaacgagaatttctggtggacgcacaagatatctgtgatgtactcagtcaagacactgtaagttatctcttatgttcgtgctccttacagtcaataaataagatttagagcatgccattttataagcaaaactaatacttgatattatataattttcagggtactcataagatattgggtataaaattgaatattgatgagattgatgaactgaatgtgcatgagaatgccttcaaagggatgcgcaatctgcgtttcctggaaattcactcacaaaaccgtcatgagtttggaaacgaagaagttagaattcacttacctgaaaacttcgactatttgcctccaaaacttaaaatattggattggtttggatatccaatgagatgtctgccttctaagtttcgtcctgaaaaactcgtcaagctcaaaatggtgaatagcaagctcgagaagctgtgggaagggattgtggtaagttttgagaatagtttgtgatgttatttgtagtaagactaatctttattttattttttggatgacaatcttgttctactgagctcatgtgttctgttcctttttttttttgttgagtacagtcgcttacatgtcttaaagagatggatatgtcgggatctacaaacttgatagaaatgccagatctttcaaaggccaccaatctggagacacttaatgttggggcttgctatagtttggtgacttttccccaaatctcaagcaccatcgtagatgtcgacatagccggaacatccattgaagaaataccttcaaatttgagtttgtgtttcgagaatctccatacctttaagatgcacagcccaaagaaactatcggaaagagtgcaggtatgtatgtagttccaaactttgtgtgtttctccaatctgttttacgttatagatattagatattggtgaaaatgaaactaaggttatattgtatttatcggagggaagaagagtagcgctgaatatgattttgtgtatttggttcagcttcttactctcctcacgccgatcatgtctccctctttgtggtatctgaatctctcggataaccctggcttggtggagcttccttcttcatttaagaatctccataaactggagagattgaaaattagaaactgcgtaaatctggaaactcttcccaccggaatcaacctcggatctctctcgagagtagatctaaggggatgctcacggttgagaacttttcctgatatctcaaccaacatcaaaaacctcgatctcagcgaaacagccattgaagagattccttgttggattgagaaattctccaggctttactccctacggatgaagggatgcaacaatttggaatatgtaaacctaaacatttctaaactcaaatatcttttcgaagtcgacttttcagactgcaagtcattgactggagctagctggaataatcgtccaagagaaagtgccttgagttattaccacagtttcgacattggtatcgatttcaccaagtgcttaaacttggatcaagaagctctgtttcaaaagaaaacatatttcggttgtcaactgaagttgtcaggtgaagaagtgccttcatatttcacgcaccgtactactggaacctcctcctctctcaccattcctttacttcacagctgtctctcacaaccattcctccgattcagggcttgcattgtgtttgattcgcacaatgagacatatagcaaatgtgtctttagattcaaaggcagttttcagaactgctctgattcctataatcaggcacaagacttctgcgcagtcacggaggattatttgatctattcatatgagaaggatggttgtctgtttgtattagactaccagatgtctcaaatccctttagaaatgaacttcgatggcctggatctgaagattcatattgttgattgttataatgctaaaataaaaggatggggtatacgaatcttagaggaggactgttcatcggcagacaaccgacttggttatccaaacattctaccacatgtttttgaagccgatgaatgcaatatgaggctggtgaatgtggaggcaaatgatgcagtgacggaaagaagcgggtaaaggcattaatcatgaacttatcacagtattttctatatcataatttcttgtactgagacttttttttctttttctgcagatttcgtgaataaagttttgattgtgttaggttgtaacgcagagcatctaaaattaggaattaagagagtttcccatccaacttgcttgtggatcttagtatgcggagaagtaagagcacaatattgtgggaaggagtagtgcatgtatgttttcttcaaccttccttccttttatactagttcttacaaaaatggttatgcctggcagatctctagaaatgaccaaacattattgtgtgtaccttaaattctcaggcagtgcctctttttctatcagagattgttcctgcacagctcaagggaggtctcaacattgtattccaactcatggtcacaattggaatcctaatagccaacctggtcaactacttcactgccaccgttcaccctaacggatcgcgaatcgccctcggtggagctgcaatccccgcggttatcctcctcttgggttcactgatcatctgtgagacccccacgagcctcatagagcgcaacaaaaacgaagaaggcagagaaactctaaggaagatcagaggagttga

SEQ ID NO: 9 - protein, 1195 aa, Brassica napus
MALSLASSPSSSRTWLYDVFPSFSGVDVRVTFLSHLLKEFDKKLITAFKDNEIERSRSLDPELKQAIKDSRIAVVIFSQNYASSSWCLNELLEIVKRGQMVIPVFYRLDPSHVRKQTGEFGKIFEETCKNQKEEVIITQWRRALTDVANTLGYHSVNWGNEAAMIEEIANDVLDKLLLTSSKDSENFVGIEDHLAELSVLLQLDAEEVRMVGLWGSSGIGKTTIARVLFQRLSRHFRGSIFIDRAFVSKTMEIFKEANPDDYNMKLHLQRNFLSEILGKGDIKINHLSAVEERLKNQKVLIFIDDFDDQVVLEALVGQTQWFGSGSRIVVVTNDKQYLRAHGINHIYEVCLPTENLAVEMLCRSAFRKKAAPEGFEELVAKVTGLAGSLPLGLNVLGSYLRGREKKYWMDLLPRLQNGLDGKIEKTLRVSYDGLTSEEDKALFRHIACLFQWKKVTYLKLLLADSGLSVTVGLENLADKSIIHVSTNYVVMHRLLEEMGRGIVRLDEPEKREFLVDAQDICDVLSQDTGTHKILGIKLNIDEIDELNVHENAFKGMRNLRFLEIHSQNRHEFGNEEVRIHLPENFDYLPPKLKILDWFGYPMRCLPSKFRPEKLVKLKMVNSKLEKLWEGIVSLTCLKEMDMSGSTNLIEMPDLSKATNLETLNVGACYSLVTFPQISSTIVDVDIAGTSIEEIPSNLSLCFENLHTFKMHSPKKLSERVQLLTLLTPIMSPSLWYLNLSDNPGLVELPSSFKNLHKLERLKIRNCVNLETLPTGINLGSLSRVDLRGCSRLRTFPDISTNIKNLDLSETAIEEIPCWIEKFSRLYSLRMKGCNNLEYVNLNISKLKYLFEVDFSDCKSLTGASWNNRPRESALSYYHSFDIGIDFTKCLNLDQEALFQKKTYFGCQLKLSGEEVPSYFTHRTTGTSSSLTIPLLHSCLSQPFLRFRACIVFDSHNETYSKCVFRFKGSFQNCSDSYNQAQDFCAVTEDYLIYSYEKDGCLFVLDYQMSQIPLEMNFDGLDLKIHIVDCYNAKIKGWGIRILEEDCSSADNRLGYPNILPHVFEADECNMRLVNVEANDAVTERSGMRRSKSTILWEGVVHAVPLFLSEIVPAQLKGGLNIVFQLMVTIGILIANLVNYFTATVHPNGSRIALGGAAIPAVILLLGSLIICETPTSLIERNKNEEGRETLRKIRG

SEQ ID NO: 10 - DNA, 8102 bp, Artificial Sequence
  nucleotide sequence of the T-DNA 35S::CRT
aattacaacggtatatatcctgccagtactttgtggcgctctatcatagctataaacctattcagcacaatatcgattaagggccccctcgagggcgatcgctacgtacctgcaggcccgggttaattaagcggccgcaacatggagtcaaaaattcagatcgaggatctaacagaactcgccgtgaagactggcgaacagttcatacagagtcttttacgactcaatgacaagaagaaaatcttcgtcaacatggtggagcacgacactctcgtctactccaagaatatcaaagatacagtctcagaagaccaaagggctattgagacttttcaacaaagggtaatatcgggaaacctcctcggattccattgcccagctatctgtcacttcatcaaaaggacagtagaaaaggaaggtggcacctacaaatgccatcattgcgataaaggaaaggctatcgttcaagatgcccctgccgacagtggtcccaaagatggacccccacccacgaggagcatcgtggaaaaagaagacgttccaaccacgtcttcaaagcaagtggattgatgtgatatctccactgacgtaagggatgacgcacaatcccactatccttcgcaagacccttcctctatataaggaagttcatttcatttggagaggactcgagctcatttctctattacttcagccataacaaaagaactcttttctcttcttattaaaccaaaaccatggctctctcattagcttcttctccttcctcttgtcgcacttggttgtacgatgttttccctagcttcagtggggtagacgttcgtgttactttcctcagccacttgttgaaggagtttgacaaaaagttgatcactgctttcaaagacaacgagatcgagagaagtcgatcactggatcccgagcttaaacaagccattaaagattcgaggatcgcagtggttatcttctcccaaaactatgcctcttcaagctggtgtcttaatgagttgttagagatagtcaagtgtggtcaaatggtgatacctgttttctaccggttggatccttcccatgtgaggaaacaaaccggtgactttggtaagttctttgaagaaacatgcaacaacaaaacagaggaagagaaaatacagtggaggagagctttgaccgatgtagccaatactctcgggtatcattcagtaaactggtacggttttatgcttcttttgaataaaggttagacttctggttgctagggggtgatattatctttcttattgttaggggtaacgaagctgcaatgattgaagaaatcgccaatgatgttttggataaactacttttaacttcatcgaaggattcagagaactttgtgggcatcgaagatcatgttgcaaaactgagtgtattgctgcagttggacgcggaggaagtgaggatggttggtttatggggttcctcagggatcggcaagactacaattgcaagagttctgtttcaacgactttctcgacacttccgaggtagcattttcatagacagggctttcgtatctaagactatggaaattttcaaggcagctaatccggacgactataacatgaagctgcatttgcaaagaaatttcctatctgaaatcttaggtaaaggagacataaagataaatcatttgagtgcagttggggagaggctgaagaatcagaaagttcttattttcattgatgattttgatgatcaagttgtgctagaagccttggttggtcaaactcaatggtttggaagtgggagcagaatcgttgtggttacaaatgataagcagtatctaagggcccatgggattaatcacatttacaaggtctgtctcccaactaaaaagctagctgttgagatgttatgtcgatctgctttcaggaaaaaggctgcacctgaaggttttgaggagcttgtagctaaagttacaggacttgctggtagtcttcctttaggtcttaatgttttgggttcatatctacggggaagggacaaggagtactggatggatttgttgccaaggcttcagaatggtttagatgggaaaattgagaagacattgagagtcagctacgatggattaacaagcgaagaagataaagcgttatttcgccatattgcatgccttttccagtgggaaaaagtcacatacctgaagttgctgctcgctgatagtgggttgagtgttacggttgggctggaaaacctagctgataagtccctcattcatgtaagagaggattatgtgaagatgcaccgtttgttagaagagatgggtagacgtattgttaggcttgacgagcctgaaaaacgagaatttctggtggacgcacaagatatctgtgatgtactcagtcaagacactgtaagttatctcttatgttcgtgctcctttcagtcaataaataagatttagagcatgccattttataagcaaaactaatacttgatattatataattttcagggtactcataagatattgggtataaaattgaatattgatgagattgatgaactgaatgtgcatgagaatgccttcaaagggatgcgcaatctgcgtttcctggaaattcactcacaaaaccgtcatgagtttggaaacgaagaagttagaattcacttacctgaaaacttcgactatttgcctcctaaacttaaaatattggattggtatgaatatccaatgagatgtctgccttctaagtttcgtcctgaaaaactcgtcaagctcaaaatggtgaatagcaagctcgagaagctgtgggaagggattgtggtaagttttgagaatagtttgtgatgttatttgtagtaagactaatctttattttattttttggatgacaatcttgttctactgagctcatgtgttctgttcctttttttttttgttgagtacagtcgcttacatgtcttaaaaagatgaatatgtcgggatctcaaaacttgatagaaatgccagatctttcaaaggccaccaatctggagacactatatcttgaggattgctttagtttggtcaagcttccttcctctattccacaccccaacaaactgacgacattaatcttgaagaactgtcgaaatgtggagactattccaattggcattagcctcaaatctcttaaaaacctacgtactgatggttgctcacggatgaggacttttccccaaatctcaagcaccatcgaagatgtctacataggcgcaacatccattgaagaaataccttcaaatttgagtttgtgtttcgagaatctccatacctttacgatgcacagcccaaagaaactatgggaaagagtgcaggtatgtatgtagttccaaactttgtgtgtttctccaatctgttttacgttatagatattagataatggtgcaaatgaaactaaggttatattgtatttatcggagggaagaagagtagcgctgaatatgattttgtgtatttggttcagcttcttactctcctcacgacgatcatgtctccctctttgtggtatctggatctctcggataaccctggcttggtggagcttccttcttcatttaagaatctccataacctgaggagattggaaattagaaactgcgtaaatctggaaactcttcccaccggaatcaacctcggatctctcaaaatcctagatctcaggggatgctcacggttgaggacttttcctgatatctcaacccacatcacacatctttatctaagcggaacagggattgaagagattccttgttcgattgagaaattctccaggcttggctccctacatatgaacggatgcaacaatttggaatatgtaaacctaaacctttttaaactcaaacatcttcacgaagtcgacttttcagactgcaagtgcttaaacttggatcaagaagctctgtttcaaaagaaaacatattcagtttgtcaactgaagttgtcaggtgaagaagtgccttcatatttcacgcaccgtactactggaacctcctcctctctcaccattcctctacttcacagctgtatctcacaatcattcctccgattcagggcttgtattgtgtttgattcggacaaggacaatgagtcatatagcagatgtgcctttagattcaaaggcagttttcggaactgctctgattcctataatcaggcacaagacttctgcgcagtcacggatgattataagatccgttcatataagaaggatggttgtctgcttgtattagactaccagatgtctcaaatccctttagaaatgaacttcgatggcctggatctgaagattcatattgattattgtcgttctgctaaaataaaaggatggggtatacgaatcttagaggaggactgttcatcggcagacaaccgacttggttatccaaacattctaccacatgtttttgaagccgatgaatgcaatgaggctggtgaatgtgggaggcaaatgatgtagtgacggaaagaagcgggtaaaggcattaatcatgaacttatcacagtattttctatatcataatttcttgtactgagacttttttttctttttctgcagatttcgtgaataaacttttgattgtgttaggttgtaacgcagagcatctaaaattaggaattaagagagattcccatccaacttgcttgtggatcttagtatgcggagaagtaagagcacaaaattgtgggaaggagtagtgcatgtatgttttcttcaaccttccttcctttatactagttcttacaaaaatggttatgcctggcagatctctagaaatgacctaacattattgtgtgtaccttaaattctcaggcagtgcctctttttctatcagagattgctcctgcacagctcaggggaggtctcaacattgtattccaactcatggtcacaattggaatcctaatagccaaccttgtcaactacttcactgccaccgttcaccctaacggatggcgaatcgccctcggtggagccgcaatccccaccgttatcctagtcttcggttcactgatcatctgcgagactcccacgagcttcatagagcgcaagtgttgaaaacgcgtggcgcgcctaagctagctatatcatcaatttatgtattacacataatatcgcactcagtctttcatctacggcaatgtaccagctgatataatcagttattgaaatatttctgaatttaaacttgcatcaataaatttatgtttttgcttggactataatacctgacttgttattttatcaataaatatttaaactatatttctttcaagatgaattcgatatcattaccctgttatccctaaagcttattaatataacttcgtatagcatacattatacgaagttatgtttcaaatttattatgtgttttttttccgtggtcgagattgtgtattattctttagttattacaagacttttagctaaaatttgaaagaatttactttaagaaaatcttaacatctgagataatttcagcaatagattatatttttcattactctagcagtatttttgcagatcaatcgcaacatatatggttgttagaaaaaatgcactatatatatatatattattttttcaattaaaagtgcatgatatataatatatatatatatatatatatgtgtgtgtgtatatggtcaaagaaattcttatacaaatatacacgaacacatatatttgacaaaatcaaagtattacactaaacaatgagttggtgcatggccaaaacaaatatgtagattaaaaattccagcctccaaaaaaaaatccaagtgttgtaaagcattatatatatatagtagatcccaaatttttgtacaattccacactgatcgaatttttaaagttgaatatctgacgtaggatttttttaatgtcttacctgaccatttactaataacattcatacgttttcatttgaaatatcctctataattatattgaatttggcacataataagaaacctaattggtgatttattttactagtaaatttctggtgatgggctttctactagaaagctctcggaaaatcttggaccaaatccatattccatgacttcgattgttaaccctattagttttcacaaacatactatcaatatcattgcaacggaaaaggtacaagtaaaacattcaatccgatagggaagtgatgtaggaggttgggaagacaggcccagaaagagatttatctgacttgttttgtgtatagttttcaatgttcataaaggaagatggagacttgagaagttttttttggactttgtttagctttgttgggcgttttttttttttgatcaataactttgttgggcttatgatttgtaatattttcgtggactctttagtttatttagacgtgctaactttgttgggcttatgacttgttgtaacatattgtaacagatgacttgatgtgcgactaatctttacacattaaacatagttctgttttttgaaagttcttattttcatttttatttgaatgttatatatttttctatatttataattctagtaaaaggcaaattttgcttttaaatgaaaaaaatatatattccacagtttcacctaatcttatgcatttagcagtacaaattcaaaaatttcccatttttattcatgaatcataccattatatattaactaaatccaaggtaaaaaaaaggtatgaaagctctatagtaagtaaaatataaattccccataaggaaagggccaagtccaccaggcaagtaaaatgagcaagcaccactccaccatcacacaatttcactcatagataacgataagattcatggaattatcttccacgtggcattattccagcggttcaagccgataagggtctcaacacctctccttaggcctttgtggccgttaccaagtaaaattaacctcacacatatccacactcaaaatccaacggtgtagatcctagtccacttgaatctcatgtatcctagaccctccgatcactccaaagcttgttctcattgttgttatcattatatatagatgaccaaagcactagaccaaacctcagtcacacaaagagtaaagaagaacaatggacccagaacgacgcccggccgacatccgccgtgccaccgaggcggacatgccggcggtctgcaccatcgtcaaccactacatcgagacaagcacggtcaacttccgtaccgagccgcaggaaccgcaggagtggacggacgacctcgtccgtctgcgggagcgctatccctggctcgtcgccgaggtggacggcgaggtcgccggcatcgcctacgcgggcccctggaaggcacgcaacgcctacgactggacggccgagtcgaccgtgtacgtctccccccgccaccagcggacgggactgggctccacgctctacacccacctgctgaagtccctggaggcacagggcttcaagagcgtggtcgctgtcatcgggctgcccaacgacccgagcgtgcgcatgcacgaggcgctcggatatgccccccgcggcatgctgcgggcggccggcttcaagcacgggaactggcatgacgtgggtttctggcagctggacttcagcctgccggtaccgccccgtccggtcctgcccgtcaccgagatctgatctcacccgtctaggatcccccgatgagctaagctagctatatcatcaatttatgtattacacataatatcgcactcagtctttcatctacggcaatgtaccagctgatataatcagttattgaaatatttctgaatttaaacttgcatcaataaatttatgtttttgcttggactataatacctgacttgttattttatcaataaatatttaaactatatttctttcaagataaacataacttcgtatagcatacattatacgaagttatcaaaacgtcgtgagacagtttggttaactataacggtcctaaggtagcgatcgaggcattacggcattacggcactcgcgagggtccgaatctatgtcgggtgcggagaaagaggtaatgaaatggcaattcgagcatggagccatttacaattgaatatatcctgccg

SEQ ID NO: 11 - DNA, 121 bp, Brassica napus
atgatctttcatcaaaatatcggatgagaaagcttgaagcttcgggactgctcatatactattaagkaaaatagtatttgtgtataaagaagtctattagttagtaaacaaattgagagaa

SEQ ID NO: 12 - DNA, 121 bp, Brassica napus
cttctggtttgatacckgttmagmaaatgtcatcggtcrgtctgatttgattgaagaaacgggtaagttgtgcagagactgtgaagctcaaggcataggcatagctagcaattattcaacc